European Patent Application EP 4 159 744 A1, published April 5, 2023. Title: A novel anti-inflammatory peptides and use thereof. Applicant: MITOQUEST. The sequence listing filed with the application follows.

SEQUENCE LISTING (63 sequences)

SEQ ID NO: 1 - protein, 8 aa, Artificial Sequence
  MQP-15
LKSLKTLH

SEQ ID NO: 2 - protein, 8 aa, Artificial Sequence
  MQP-23
LQHLEDGM

SEQ ID NO: 3 - protein, 6 aa, Artificial Sequence
  MQP-31
DGTECR

SEQ ID NO: 4 - protein, 9 aa, Artificial Sequence
  MQP-37
SLVLADARW

SEQ ID NO: 5 - protein, 9 aa, Artificial Sequence
  MQP-37A1
ALVLADARW

SEQ ID NO: 6 - protein, 9 aa, Artificial Sequence
  MQP-37A2
SAVLADARW

SEQ ID NO: 7 - protein, 9 aa, Artificial Sequence
  MQP-37A3
SLALADARW

SEQ ID NO: 8 - protein, 9 aa, Artificial Sequence
  MQP-37A4
SLVAADARW

SEQ ID NO: 9 - protein, 9 aa, Artificial Sequence
  MQP-37A6
SLVLAAARW

SEQ ID NO: 10 - protein, 9 aa, Artificial Sequence
  MQP-37A8
SLVLADAAW

SEQ ID NO: 11 - protein, 9 aa, Artificial Sequence
  MQP-37A9
SLVLADARA

SEQ ID NO: 12 - protein, 9 aa, Artificial Sequence
  MQP-37S1C
CLVLAAARW

SEQ ID NO: 13 - protein, 9 aa, Artificial Sequence
  MQP-37S1D
DLVLAAARW

SEQ ID NO: 14 - protein, 9 aa, Artificial Sequence
  MQP-37S1E
ELVLAAARW

SEQ ID NO: 15 - protein, 9 aa, Artificial Sequence
  MQP-37S1F
FLVLAAARW

SEQ ID NO: 16 - protein, 9 aa, Artificial Sequence
  MQP-37S1G
GLVLAAARW

SEQ ID NO: 17 - protein, 9 aa, Artificial Sequence
  MQP-37S1H
HLVLAAARW

SEQ ID NO: 18 - protein, 9 aa, Artificial Sequence
  MQP-37S1I
ILVLAAARW

SEQ ID NO: 19 - protein, 9 aa, Artificial Sequence
  MQP-37S1K
KLVLAAARW

SEQ ID NO: 20 - protein, 9 aa, Artificial Sequence
  MQP-37S1L
LLVLAAARW

SEQ ID NO: 21 - protein, 9 aa, Artificial Sequence
  MQP-37S1M
MLVLAAARW

SEQ ID NO: 22 - protein, 9 aa, Artificial Sequence
  MQP-37S1N
NLVLAAARW

SEQ ID NO: 23 - protein, 9 aa, Artificial Sequence
  MQP-37S1P
PLVLAAARW

SEQ ID NO: 24 - protein, 9 aa, Artificial Sequence
  MQP-37S1Q
QLVLAAARW

SEQ ID NO: 25 - protein, 9 aa, Artificial Sequence
  MQP-37S1R
RLVLAAARW

SEQ ID NO: 26 - protein, 9 aa, Artificial Sequence
  MQP-37S1T
TLVLAAARW

SEQ ID NO: 27 - protein, 9 aa, Artificial Sequence
  MQP-37S1V
VLVLAAARW

SEQ ID NO: 28 - protein, 9 aa, Artificial Sequence
  MQP-37S1W
WLVLAAARW

SEQ ID NO: 29 - protein, 9 aa, Artificial Sequence
  MQP-37S1Y
YLVLAAARW

SEQ ID NO: 30 - protein, 9 aa, Artificial Sequence
  MQP-37D6C
SLVLACARW

SEQ ID NO: 31 - protein, 9 aa, Artificial Sequence
  MQP-37D6E
SLVLAEARW

SEQ ID NO: 32 - protein, 9 aa, Artificial Sequence
  MQP-37D6F
SLVLAFARW

SEQ ID NO: 33 - protein, 9 aa, Artificial Sequence
  MQP-37D6G
SLVLAGARW

SEQ ID NO: 34 - protein, 9 aa, Artificial Sequence
  MQP-37D6H
SLVLAHARW

SEQ ID NO: 35 - protein, 9 aa, Artificial Sequence
  MQP-37D6I
SLVLAIARW

SEQ ID NO: 36 - protein, 9 aa, Artificial Sequence
  MQP-37D6K
SLVLAKARW

SEQ ID NO: 37 - protein, 9 aa, Artificial Sequence
  MQP-37D6L
SLVLALARW

SEQ ID NO: 38 - protein, 9 aa, Artificial Sequence
  MQP-37D6M
SLVLAMARW

SEQ ID NO: 39 - protein, 9 aa, Artificial Sequence
  MQP-37D6N
SLVLANARW

SEQ ID NO: 40 - protein, 9 aa, Artificial Sequence
  MQP-37D6P
SLVLAPARW

SEQ ID NO: 41 - protein, 9 aa, Artificial Sequence
  MQP-37D6Q
SLVLAQARW

SEQ ID NO: 42 - protein, 9 aa, Artificial Sequence
  MQP-37D6R
SLVLARARW

SEQ ID NO: 43 - protein, 9 aa, Artificial Sequence
  MQP-37D6S
SLVLASARW

SEQ ID NO: 44 - protein, 9 aa, Artificial Sequence
  MQP-37D6T
SLVLATARW

SEQ ID NO: 45 - protein, 9 aa, Artificial Sequence
  MQP-37D6V
SLVLAVARW

SEQ ID NO: 46 - protein, 9 aa, Artificial Sequence
  MQP-37D6W
SLVLAWARW

SEQ ID NO: 47 - protein, 9 aa, Artificial Sequence
  MQP-37D6Y
SLVLAYARW

SEQ ID NO: 48 - protein, 10 aa, Artificial Sequence
  MQP-Y9
KRLLFWIFIK

SEQ ID NO: 49 - protein, 7 aa, Artificial Sequence
  MQP-91
QMVSMVG

SEQ ID NO: 50 - protein, 12 aa, Artificial Sequence
  MQP-T234
KVGDRARWGSRS

SEQ ID NO: 51 - protein, 10 aa, Artificial Sequence
  MQP-S442
LERQSRSWRN

SEQ ID NO: 52 - protein, 10 aa, Artificial Sequence
  MQP-341
EWLGRGRFNG

SEQ ID NO: 53 - protein, 10 aa, Artificial Sequence
  MQP-Y9A1
ARLLFWIFIK

SEQ ID NO: 54 - protein, 10 aa, Artificial Sequence
  MQP-Y9A2
KALLFWIFIK

SEQ ID NO: 55 - protein, 10 aa, Artificial Sequence
  MQP-Y9A3
KRALFWIFIK

SEQ ID NO: 56 - protein, 10 aa, Artificial Sequence
  MQP-Y9A4
KRLAFWIFIK

SEQ ID NO: 57 - protein, 10 aa, Artificial Sequence
  MQP-Y9A5
KRLLAWIFIK

SEQ ID NO: 58 - protein, 10 aa, Artificial Sequence
  MQP-Y9A6
KRLLFAIFIK

SEQ ID NO: 59 - protein, 10 aa, Artificial Sequence
  MQP-Y9A7
KRLLFWAFIK

SEQ ID NO: 60 - protein, 10 aa, Artificial Sequence
  MQP-Y9A8
KRLLFWIAIK

SEQ ID NO: 61 - protein, 10 aa, Artificial Sequence
  MQP-Y9A9
KRLLFWIFAK

SEQ ID NO: 62 - protein, 10 aa, Artificial Sequence
  MQP-Y9A10
KRLLFWIFIA

SEQ ID NO: 63 - protein, 9 aa, Artificial Sequence
  MQP-37S1A
ALVLAAARW